European Patent Specification EP 3 689 371 B1, published October 22, 2025. Title: PROTEINS SPECIFIC FOR BAFF AND B7RP1 AND USES THEREOF. Applicant: Amgen Inc. Application not yet assigned. The sequence listing filed with the application follows.

SEQUENCE LISTING (72 sequences)

SEQ ID NO: 1 - protein, 18 aa, Artificial Sequence
  source: /note="Description of Artificial Sequence: Synthetic peptide"
LPGCKWDLLIKQWVCDPL

SEQ ID NO: 2 - protein, 18 aa, Artificial Sequence
  source: /note="Description of Artificial Sequence: Synthetic peptide"
FHDCKWDLLTKQWVCHGL

SEQ ID NO: 3 - protein, 12 aa, Artificial Sequence
  source: /note="Description of Artificial Sequence: Synthetic peptide"
  VARIANT (3)..(3): /replace="Tyr" or "Phe"
  MOD_RES (5)..(5): Any amino acid
  VARIANT (7)..(7): /replace="Ile"
  VARIANT (8)..(8): /replace="Arg" or "His"
  VARIANT (10)..(10): /replace="Arg" or "His" or "Ala" or "Val" or "Leu" or "Ile" or "Pro" or "Phe" or "Trp" or "Met"
  misc_feature (1)..(12): /note="Variant residues given in the sequence have no preference with respect to those in the annotations for variant positions"
CKWDXLTKQKVC

SEQ ID NO: 4 - protein, 4 aa, Artificial Sequence
  source: /note="Description of Artificial Sequence: Synthetic peptide"
GGGG

SEQ ID NO: 5 - protein, 23 aa, Artificial Sequence
  source: /note="Description of Artificial Sequence: Synthetic peptide"
  VARIANT (12)..(12): /replace="Val"
  misc_feature (1)..(23): /note="Variant residues given in the sequence have no preference with respect to those in the annotations for variant positions"
GSGSATGGSGSSASSGSGSATHL

SEQ ID NO: 6 - protein, 23 aa, Artificial Sequence
  source: /note="Description of Artificial Sequence: Synthetic peptide"
GSGSATGGSGSVASSGSGSATHL

SEQ ID NO: 7 - protein, 23 aa, Artificial Sequence
  source: /note="Description of Artificial Sequence: Synthetic peptide"
GSGSATGGSGSSASSGSGSATHL

SEQ ID NO: 8 - protein, 11 aa, Artificial Sequence
  source: /note="Description of Artificial Sequence: Synthetic peptide"
RASQGISNWLA

SEQ ID NO: 9 - protein, 7 aa, Artificial Sequence
  source: /note="Description of Artificial Sequence: Synthetic peptide"
AASSLQS

SEQ ID NO: 10 - protein, 9 aa, Artificial Sequence
  source: /note="Description of Artificial Sequence: Synthetic peptide"
QQYDSYPRT

SEQ ID NO: 11 - protein, 5 aa, Artificial Sequence
  source: /note="Description of Artificial Sequence: Synthetic peptide"
SYWMS

SEQ ID NO: 12 - protein, 17 aa, Artificial Sequence
  source: /note="Description of Artificial Sequence: Synthetic peptide"
YIKQDGNEKYYVDSVKG

SEQ ID NO: 13 - protein, 12 aa, Artificial Sequence
  source: /note="Description of Artificial Sequence: Synthetic peptide"
EGILWFGDLPTF

SEQ ID NO: 14 - protein, 108 aa, Artificial Sequence
  source: /note="Description of Artificial Sequence: Synthetic polypeptide"
DIQMTQSPSSLSASVGDRVTITCRASQGISNWLAWYQQKPEKAPKSLIYAASSLQSGVPSRFSGSGSGTDFTLTISSLQPEDFATYYCQQYDSYPRTFGQGTKVEIKR

SEQ ID NO: 15 - protein, 121 aa, Artificial Sequence
  source: /note="Description of Artificial Sequence: Synthetic polypeptide"
EVQLVESGGGLVQPGGSLRLSCAASGFTFSSYWMSWVRQAPGKGLEWVAYIKQDGNEKYYVDSVKGRFTISRDNAKNSLYLQMNSLRAEDTAVYYCAREGILWFGDLPTFWGQGTLVTVSS

SEQ ID NO: 16 - protein, 509 aa, Artificial Sequence
  source: /note="Description of Artificial Sequence: Synthetic polypeptide"
EVQLVESGGGLVQPGGSLRLSCAASGFTFSSYWMSWVRQAPGKGLEWVAYIKQDGNEKYYVDSVKGRFTISRDNAKNSLYLQMNSLRAEDTAVYYCAREGILWFGDLPTFWGQGTLVTVSSASTKGPSVFPLAPCSRSTSESTAALGCLVKDYFPEPVTVSWNSGALTSGVHTFPAVLQSSGLYSLSSVVTVPSSNFGTQTYTCNVDHKPSNTKVDKTVERKCCVECPPCPAPPVAGPSVFLFPPKPKDTLMISRTPEVTCVVVDVSHEDPEVQFNWYVDGVEVHNAKTKPREEQFNSTFRVVSVLTVVHQDWLNGKEYKCKVSNKGLPAPIEKTISKTKGQPREPQVYTLPPSREEMTKNQVSLTCLVKGFYPSDIAVEWESNGQPENNYKTTPPMLDSDGSFFLYSKLTVDKSRWQQGNVFSCSVMHEALHNHYTQKSLSLSPGGGGGLPGCKWDLLIKQWVCDPLGSGSATGGSGSGASSGSGSATGSLPGCKWDLLIKQWVCDPL

SEQ ID NO: 17 - protein, 511 aa, Artificial Sequence
  source: /note="Description of Artificial Sequence: Synthetic polypeptide"
EVQLVESGGGLVQPGGSLRLSCAASGFTFSSYWMSWVRQAPGKGLEWVAYIKQDGNEKYYVDSVKGRFTISRDNAKNSLYLQMNSLRAEDTAVYYCAREGILWFGDLPTFWGQGTLVTVSSASTKGPSVFPLAPCSRSTSESTAALGCLVKDYFPEPVTVSWNSGALTSGVHTFPAVLQSSGLYSLSSVVTVPSSNFGTQTYTCNVDHKPSNTKVDKTVERKCCVECPPCPAPPVAGPSVFLFPPKPKDTLMISRTPEVTCVVVDVSHEDPEVQFNWYVDGVEVHNAKTKPREEQFNSTFRVVSVLTVVHQDWLNGKEYKCKVSNKGLPAPIEKTISKTKGQPREPQVYTLPPSREEMTKNQVSLTCLVKGFYPSDIAVEWESNGQPENNYKTTPPMLDSDGSFFLYSKLTVDKSRWQQGNVFSCSVMHEALHNHYTQKSLSLSPGKGGGGGLPGCKWDLLIKQWVCDPLGSGSATGGSGSVASSGSGSATHLLPGCKWDLLIKQWVCDPL

SEQ ID NO: 18 - protein, 511 aa, Artificial Sequence
  source: /note="Description of Artificial Sequence: Synthetic polypeptide"
EVQLVESGGGLVQPGGSLRLSCAASGFTFSSYWMSWVRQAPGKGLEWVAYIKQDGNEKYYVDSVKGRFTISRDNAKNSLYLQMNSLRAEDTAVYYCAREGILWFGDLPTFWGQGTLVTVSSASTKGPSVFPLAPCSRSTSESTAALGCLVKDYFPEPVTVSWNSGALTSGVHTFPAVLQSSGLYSLSSVVTVPSSNFGTQTYTCNVDHKPSNTKVDKTVERKCCVECPPCPAPPVAGPSVFLFPPKPKDTLMISRTPEVTCVVVDVSHEDPEVQFNWYVDGVEVHNAKTKPREEQFNSTFRVVSVLTVVHQDWLNGKEYKCKVSNKGLPAPIEKTISKTKGQPREPQVYTLPPSREEMTKNQVSLTCLVKGFYPSDIAVEWESNGQPENNYKTTPPMLDSDGSFFLYSKLTVDKSRWQQGNVFSCSVMHEALHNHYTQKSLSLSPGKGGGGGLPGCKWDLLIKQWVCDPLGSGSATGGSGSSASSGSGSATHLLPGCKWDLLIKQWVCDPL

SEQ ID NO: 19 - protein, 214 aa, Artificial Sequence [sequence omitted]

SEQ ID NO: 20 - protein, 9 aa, Artificial Sequence
  source: /note="Description of Artificial Sequence: Synthetic peptide"
  MOD_RES (2)..(9): Any amino acid
CXXXXXXXX

SEQ ID NO: 21 - protein, 5 aa, Artificial Sequence
  source: /note="Description of Artificial Sequence: Synthetic peptide"
LEWIG

SEQ ID NO: 22 - protein, 4 aa, Artificial Sequence
  source: /note="Description of Artificial Sequence: Synthetic peptide"
  MOD_RES (3)..(3): Any amino acid
WGXG

SEQ ID NO: 23 - protein, 4 aa, Artificial Sequence
  source: /note="Description of Artificial Sequence: Synthetic peptide"
  MOD_RES (3)..(3): Any amino acid
FGXG

SEQ ID NO: 24 - protein, 23 aa, Artificial Sequence
  source: /note="Description of Artificial Sequence: Synthetic peptide"
GSGSATGGSGSGASSGSGSATGS

SEQ ID NO: 25 - protein, 447 aa, Artificial Sequence
  source: /note="Description of Artificial Sequence: Synthetic polypeptide"
EVQLVESGGGLVQPGGSLRLSCAASGFTFSSYWMSWVRQAPGKGLEWVAYIKQDGNEKYYVDSVKGRFTISRDNAKNSLYLQMNSLRAEDTAVYYCAREGILWFGDLPTFWGQGTLVTVSSASTKGPSVFPLAPCSRSTSESTAALGCLVKDYFPEPVTVSWNSGALTSGVHTFPAVLQSSGLYSLSSVVTVPSSNFGTQTYTCNVDHKPSNTKVDKTVERKCCVECPPCPAPPVAGPSVFLFPPKPKDTLMISRTPEVTCVVVDVSHEDPEVQFNWYVDGVEVHNAKTKPREEQFNSTFRVVSVLTVVHQDWLNGKEYKCKVSNKGLPAPIEKTISKTKGQPREPQVYTLPPSREEMTKNQVSLTCLVKGFYPSDIAVEWESNGQPENNYKTTPPMLDSDGSFFLYSKLTVDKSRWQQGNVFSCSVMHEALHNHYTQKSLSLSPGK

SEQ ID NO: 26 - protein, 508 aa, Artificial Sequence
  source: /note="Description of Artificial Sequence: Synthetic polypeptide"
LPGCKWDLLIKQWVCDPLGSGSATGGSGSGASSGSGSATGSLPGCKWDLLIKQWVCDPLGGEVQLVESGGGLVQPGGSLRLSCAASGFTFSSYWMSWVRQAPGKGLEWVAYIKQDGNEKYYVDSVKGRFTISRDNAKNSLYLQMNSLRAEDTAVYYCAREGILWFGDLPTFWGQGTLVTVSSASTKGPSVFPLAPCSRSTSESTAALGCLVKDYFPEPVTVSWNSGALTSGVHTFPAVLQSSGLYSLSSVVTVPSSNFGTQTYTCNVDHKPSNTKVDKTVERKCCVECPPCPAPPVAGPSVFLFPPKPKDTLMISRTPEVTCVVVDVSHEDPEVQFNWYVDGVEVHNAKTKPREEQFNSTFRVVSVLTVVHQDWLNGKEYKCKVSNKGLPAPIEKTISKTKGQPREPQVYTLPPSREEMTKNQVSLTCLVKGFYPSDIAVEWESNGQPENNYKTTPPMLDSDGSFFLYSKLTVDKSRWQQGNVFSCSVMHEALHNHYTQKSLSLSPGK

SEQ ID NO: 27 - protein, 275 aa, Artificial Sequence
  source: /note="Description of Artificial Sequence: Synthetic polypeptide"
LPGCKWDLLIKQWVCDPLGSGSATGGSGSGASSGSGSATGSLPGCKWDLLIKQWVCDPLGGDIQMTQSPSSLSASVGDRVTITCRASQGISNWLAWYQQKPEKAPKSLIYAASSLQSGVPSRFSGSGSGTDFTLTISSLQPEDFATYYCQQYDSYPRTFGQGTKVEIKRTVAAPSVFIFPPSDEQLKSGTASVVCLLNNFYPREAKVQWKVDNALQSGNSQESVTEQDSKDSTYSLSSTLTLSKADYEKHKVYACEVTHQGLSSPVTKSFNRGEC

SEQ ID NO: 28 - protein, 511 aa, Artificial Sequence
  source: /note="Description of Artificial Sequence: Synthetic polypeptide"
EVQLVESGGGLVQPGGSLRLSCAASGFTFSSYWMSWVRQAPGKGLEWVAYIKQDGNEKYYVDSVKGRFTISRDNAKNSLYLQMNSLRAEDTAVYYCAREGILWFGDLPTFWGQGTLVTVSSASTKGPSVFPLAPCSRSTSESTAALGCLVKDYFPEPVTVSWNSGALTSGVHTFPAVLQSSGLYSLSSVVTVPSSNFGTQTYTCNVDHKPSNTKVDKTVERKCCVECPPCPAPPVAGPSVFLFPPKPKDTLMISRTPEVTCVVVDVSHEDPEVQFNWYVDGVEVHNAKTKPREEQFNSTFRVVSVLTVVHQDWLNGKEYKCKVSNKGLPAPIEKTISKTKGQPREPQVYTLPPSREEMTKNQVSLTCLVKGFYPSDIAVEWESNGQPENNYKTTPPMLDSDGSFFLYSKLTVDKSRWQQGNVFSCSVMHEALHNHYTQKSLSLSPGGGGGLPGCKWDLLIKQWVCDPLGGGGSGGGGSGGGGSGGGGSGGGGSLPGCKWDLLIKQWVCDPL

SEQ ID NO: 29 - protein, 510 aa, Artificial Sequence
  source: /note="Description of Artificial Sequence: Synthetic polypeptide"
EVQLVESGGGLVQPGGSLRLSCAASGFTFSSYWMSWVRQAPGKGLEWVAYIKQDGNEKYYVDSVKGRFTISRDNAKNSLYLQMNSLRAEDTAVYYCAREGILWFGDLPTFWGQGTLVTVSSASTKGPSVFPLAPCSRSTSESTAALGCLVKDYFPEPVTVSWNSGALTSGVHTFPAVLQSSGLYSLSSVVTVPSSNFGTQTYTCNVDHKPSNTKVDKTVERKCCVECPPCPAPPVAGPSVFLFPPKPKDTLMISRTPEVTCVVVDVSHEDPEVQFNWYVDGVEVHNAKTKPREEQFNSTFRVVSVLTVVHQDWLNGKEYKCKVSNKGLPAPIEKTISKTKGQPREPQVYTLPPSREEMGGLPGCKWDLLIKQWVCDPLGSGSATGGSGSGASSGSGSATGSLPGCKWDLLIKQWVCDPLGGTKNQVSLTCLVKGFYPSDIAVEWESNGQPENNYKTTPPMLDSDGSFFLYSKLTVDKSRWQQGNVFSCSVMHEALHNHYTQKSLSLSPGK

SEQ ID NO: 30 - protein, 490 aa, Artificial Sequence
  source: /note="Description of Artificial Sequence: Synthetic polypeptide"
EVQLVESGGGLVQPGGSLRLSCAASGFTFSSYWMSWVRQAPGKGLEWVAYIKQDGNEKYYVDSVKGRFTISRDNAKNSLYLQMNSLRAEDTAVYYCAREGILWFGDLPTFWGQGTLVTVSSASTKGPSVFPLAPCSRSTSESTAALGCLVKDYFPEPVTVSWNSGALTSGVHTFPAVLQSSGLYSLSSVVTVPSSNFGTQTYTCNVDHKPSNTKVDKTVERKCCVECPPCPAPPVAGPSVFLFPPKPKDTLMISRTPEVTCVVVDVSHEDPEVQFNWYVDGVEVHNAKTKPREEQFNSTFRVVSVLTVVHQDWLNGKEYKCKVSNKGLPAPIEKTISKTKGQPREPQVYTLPPSREEMGGLPGCKWDLLIKQWVCDPLGGTKNQVSLTCLVKGFYPSDIAVEWESNGQPENNYKTTPPMLDSDGSFFLYSKLTVDKSRWQQGNVFSCSVMHEALHNHYTQKSLSLSPGGGGGLPGCKWDLLIKQWVCDPL

SEQ ID NO: 31 - protein, 491 aa, Artificial Sequence
  source: /note="Description of Artificial Sequence: Synthetic polypeptide"
EVQLVESGGGLVQPGGSLRLSCAASGFTFSSYWMSWVRQAPGKGLEWVAYIKQDGNEKYYVDSVKGRFTISRDNAKNSLYLQMNSLRAEDTAVYYCAREGILWFGDLPTFWGQGTLVTVSSASTKGPSVFPLAPCSRSTSESTAALGCLVKDYFPEPVTVSWNSGALTSGVHTFPAVLQSSGLYSLSSVVTVPSSNFGTQTYTCNVDHKPSNTKVDKTVERKCCVECPPCPAPPVAGPSVFLFPPKPKDTLMISRTPEVTCVVVDVSHGGLPGCKWDLLIKQWVCDPLGGEDPEVQFNWYVDGVEVHNAKTKPREEQFNSTFRVVSVLTVVHQDWLNGKEYKCKVSNKGLPAPIEKTISKTKGQPREPQVYTLPPSREEMGGLPGCKWDLLIKQWVCDPLGGTKNQVSLTCLVKGFYPSDIAVEWESNGQPENNYKTTPPMLDSDGSFFLYSKLTVDKSRWQQGNVFSCSVMHEALHNHYTQKSLSLSPGK

SEQ ID NO: 32 - protein, 293 aa, Artificial Sequence
  source: /note="Description of Artificial Sequence: Synthetic polypeptide"
MLPGCKWDLLIKQWVCDPLGSGSATGGSGSTASSGSGSATHMLPGCKWDLLIKQWVCDPLGGGGGVDKTHTCPPCPAPELLGGPSVFLFPPKPKDTLMISRTPEVTCVVVDVSHEDPEVKFNWYVDGVEVHNAKTKPREEQYNSTYRVVSVLTVLHQDWLNGKEYKCKVSNKALPAPIEKTISKAKGQPREPQVYTLPPSRDELTKNQVSLTCLVKGFYPSDIAVEWESNGQPENNYKTTPPVLDSDGSFFLYSKLTVDKSRWQQGNVFSCSVMHEALHNHYTQKSLSLSPGK

SEQ ID NO: 33 - protein, 232 aa, Homo sapiens
EPKSCDKTHTCPPCPAPELLGGPSVFLFPPKPKDTLMISRTPEVTCVVVDVSHEDPEVKFNWYVDGVEVHNAKTKPREEQYNSTYRVVSVLTVLHQDWLNGKEYKCKVSNKALPAPIEKTISKAKGQPREPQVYTLPPSRDELTKNQVSLTCLVKGFYPSDIAVEWESNGQPENNYKTTPPVLDSDGSFFLYSKLTVDKSRWQQGNVFSCSVMHEALHNHYTQKSLSLSPGK

SEQ ID NO: 34 - protein, 228 aa, Homo sapiens
ERKCCVECPPCPAPPVAGPSVFLFPPKPKDTLMISRTPEVTCVVVDVSHEDPEVQFNWYVDGMEVHNAKTKPREEQFNSTFRVVSVLTVVHQDWLNGKEYKCKVSNKGLPAPIEKTISKTKGQPREPQVYTLPPSREEMTKNQVSLTCLVKGFYPSDIAVEWESNGQPENNYKTTPPMLDSDGSFFLYSKLTVDKSRWQQGNVFSCSVMHEALHNHYTQKSLSLSPGK

SEQ ID NO: 35 - protein, 279 aa, Homo sapiens
ELKTPLGDTTHTCPRCPEPKSCDTPPPCPRCPEPKSCDTPPPCPRCPEPKSCDTPPPCPRCPAPELLGGPSVFLFPPKPKDTLMISRTPEVTCVVVDVSHEDPEVQFKWYVDGVEVHNAKTKPREEQYNSTFRVVSVLTVLHQDWLNGKEYKCKVSNKALPAPIEKTISKTKGQPREPQVYTLPPSREEMTKNQVSLTCLVKGFYPSDIAVEWESSGQPENNYNTTPPMLDSDGSFFLYSKLTVDKSRWQQGNIFSCSVMHEALHNRFTQKSLSLSPGK

SEQ ID NO: 36 - protein, 229 aa, Homo sapiens
ESKYGPPCPSCPAPEFLGGPSVFLFPPKPKDTLMISRTPEVTCVVVDVSQEDPEVQFNWYVDGVEVHNAKTKPREEQFNSTYRVVSVLTVLHQDWLNGKEYKCKVSNKGLPSSIEKTISKAKGQPREPQVYTLPPSQEEMTKNQVSLTCLVKGFYPSDIAVEWESNGQPENNYKTTPPVLDSDGSFFLYSRLTVDKSRWQEGNVFSCSVMHEALHNHYTQKSLSLSLGK

SEQ ID NO: 37 - protein, 4 aa, Artificial Sequence
  source: /note="Description of Artificial Sequence: Synthetic peptide"
GGGS

SEQ ID NO: 38 - protein, 4 aa, Artificial Sequence
  source: /note="Description of Artificial Sequence: Synthetic peptide"
GGGP

SEQ ID NO: 39 - protein, 4 aa, Artificial Sequence
  source: /note="Description of Artificial Sequence: Synthetic peptide"
GGGQ

SEQ ID NO: 40 - protein, 5 aa, Artificial Sequence
  source: /note="Description of Artificial Sequence: Synthetic peptide"
GGGGG

SEQ ID NO: 41 - DNA, 54 bp, Artificial Sequence
  source: /note="Description of Artificial Sequence: Synthetic oligonucleotide"
ctgccgggttgtaaatgggacctgctgatcaaacagtgggtttgtgacccgctg

SEQ ID NO: 42 - DNA, 12 bp, Artificial Sequence
  source: /note="Description of Artificial Sequence: Synthetic oligonucleotide"
ggtggtggtggt

SEQ ID NO: 43 - DNA, 69 bp, Artificial Sequence
  source: /note="Description of Artificial Sequence: Synthetic oligonucleotide"
  modified_base (36)..(36): a, c, t, g, unknown or other
ggatccggttctgctactggtggttccggctccdbngcaagctctggttcaggcagtgcgactcatctg

SEQ ID NO: 44 - DNA, 69 bp, Artificial Sequence
  source: /note="Description of Artificial Sequence: Synthetic oligonucleotide"
ggatccggttctgctactggtggttccggctccgtcgcaagctctggttcaggcagtgcgactcatctg

SEQ ID NO: 45 - DNA, 69 bp, Artificial Sequence
  source: /note="Description of Artificial Sequence: Synthetic oligonucleotide"
ggatccggttctgctactggtggttccggctcctcggcaagctctggttcaggcagtgcgactcatctg

SEQ ID NO: 46 - DNA, 33 bp, Artificial Sequence
  source: /note="Description of Artificial Sequence: Synthetic oligonucleotide"
cgggcgagtcagggtattagcaactggttagcc

SEQ ID NO: 47 - DNA, 21 bp, Artificial Sequence
  source: /note="Description of Artificial Sequence: Synthetic oligonucleotide"
gctgcatccagtttgcaaagt

SEQ ID NO: 48 - DNA, 27 bp, Artificial Sequence
  source: /note="Description of Artificial Sequence: Synthetic oligonucleotide"
caacagtatgatagttaccctcggacg

SEQ ID NO: 49 - DNA, 15 bp, Artificial Sequence
  source: /note="Description of Artificial Sequence: Synthetic oligonucleotide"
agttattggatgagt

SEQ ID NO: 50 - DNA, 51 bp, Artificial Sequence
  source: /note="Description of Artificial Sequence: Synthetic oligonucleotide"
tacataaagcaagatggaaatgagaaatactatgtggactctgtgaagggc

SEQ ID NO: 51 - DNA, 36 bp, Artificial Sequence
  source: /note="Description of Artificial Sequence: Synthetic oligonucleotide"
gaagggatactttggttcggggacttaccgacgttc

SEQ ID NO: 52 - DNA, 324 bp, Artificial Sequence
  source: /note="Description of Artificial Sequence: Synthetic polynucleotide"
gacatccagatgacccagtctccatcctcactgtctgcatctgtaggagacagagtcaccatcacttgtcgggcgagtcagggtattagcaactggttagcctggtatcagcagaaaccagagaaagcccctaagtccctgatctatgctgcatccagtttgcaaagtggggtcccatcaaggttcagcggcagtggatctgggacagatttcactctcaccatcagcagcctgcagcctgaagattttgcaacttattactgccaacagtatgatagttaccctcggacgttcggccaagggaccaaggtggaaatcaaacga

SEQ ID NO: 53 - DNA, 363 bp, Artificial Sequence
  source: /note="Description of Artificial Sequence: Synthetic polynucleotide"
gaggtgcagctggtggagtctgggggaggcttggtccagcctggggggtccctgagactctcctgtgcagcttctggatttacctttagtagttattggatgagttgggtccgccaggctccagggaaagggctggagtgggtggcctacataaagcaagatggaaatgagaaatactatgtggactctgtgaagggccgattcaccatctccagagacaacgccaagaactcattgtatctgcaaatgaacagcctgagagccgaggacacggctgtgtattactgtgcgagggaagggatactttggttcggggacttaccgacgttctggggccagggaaccctggtcaccgtctctagt

SEQ ID NO: 54 - DNA, 1527 bp, Artificial Sequence
  source: /note="Description of Artificial Sequence: Synthetic polynucleotide"
gaggtgcagctggtggagtctgggggaggcttggtccagcctggggggtccctgagactctcctgtgcagcttctggatttacctttagtagttattggatgagttgggtccgccaggctccagggaaagggctggagtgggtggcctacataaagcaagatggaaatgagaaatactatgtggactctgtgaagggccgattcaccatctccagagacaacgccaagaactcattgtatctgcaaatgaacagcctgagagccgaggacacggctgtgtattactgtgcgagggaagggatactttggttcggggacttaccgacgttctggggccagggaaccctggtcaccgtctctagtgcctccaccaagggcccatcggtcttccccctggcgccctgctccaggagcacctccgagagcacagcggccctgggctgcctggtcaaggactacttccccgaaccggtgacggtgtcgtggaactcaggcgctctgaccagcggcgtgcacaccttcccagctgtcctacagtcctcaggactctactccctcagcagcgtggtaacggtgccctcctcaaatttcgggacgcagacatatacatgcaatgtggatcataagccttccaacacgaaggtggacaagactgtggagcggaagtgttgcgtcgagtgcccaccgtgtcccgctcctccggtcgctggcccatcagtatttctcttccctcccaagccaaaagatacactcatgatctcaagaaccccagaagtgacttgtgtggtcgtggacgtgtcgcatgaggatccggaggtgcagtttaactggtatgtggatggcgtagaagtccacaacgccaagaccaagcctagagaggaacaattcaactcgacgttcagggtggtcagcgtgttgacagtagtccaccaggactggcttaatgggaaggaatacaaatgtaaggtctcaaacaaagggctcccggcacccattgagaagacaatttccaaaaccaagggacagcccagggaaccccaagtgtatacgctgcccccaagccgggaggaaatgacgaaaaatcaggtcagcctcacgtgtctcgtaaagggattttacccgtcggacatcgcggtggagtgggagtcaaatggacagcccgaaaacaactataagaccacaccaccgatgctcgactccgacggaagcttctttttgtactcgaaactgacggtggacaaatcgcgctggcaacaggggaatgtctttagctgctcggtcatgcacgaggccctccacaatcattacactcagaaaagcttgtcgctctcgccgggtgggggtggaggactgcccggttgcaaatgggatctgttgatcaaacagtgggtatgcgaccctttgggaagcggctcggcgacgggtgggtcggggtcgggtgcgtccagcggatcgggctcggccactgggtcactccctggatgcaagtgggatcttcttatcaagcaatgggtgtgcgatcccctc

SEQ ID NO: 55 - DNA, 1533 bp, Artificial Sequence
  source: /note="Description of Artificial Sequence: Synthetic polynucleotide"
gaggtgcagctggtggagtctgggggaggcttggtccagcctggggggtccctgagactctcctgtgcagcttctggatttacctttagtagttattggatgagttgggtccgccaggctccagggaaagggctggagtgggtggcctacataaagcaagatggaaatgagaaatactatgtggactctgtgaagggccgattcaccatctccagagacaacgccaagaactcattgtatctgcaaatgaacagcctgagagccgaggacacggctgtgtattactgtgcgagggaagggatactttggttcggggacttaccgacgttctggggccagggaaccctggtcaccgtctctagtgcctccaccaagggcccatcggtcttccccctggcgccctgctccaggagcacctccgagagcacagcggccctgggctgcctggtcaaggactacttccccgaaccggtgacggtgtcgtggaactcaggcgctctgaccagcggcgtgcacaccttcccagctgtcctacagtcctcaggactctactccctcagcagcgtggtaacggtgccctcctcaaatttcgggacgcagacatatacatgcaatgtggatcataagccttccaacacgaaggtggacaagactgtggagcggaagtgttgcgtcgagtgcccaccgtgtcccgctcctccggtcgctggcccatcagtatttctcttccctcccaagccaaaagatacactcatgatctcaagaaccccagaagtgacttgtgtggtcgtggacgtgtcgcatgaggatccggaggtgcagtttaactggtatgtggatggcgtagaagtccacaacgccaagaccaagcctagagaggaacaattcaactcgacgttcagggtggtcagcgtgttgacagtagtccaccaggactggcttaatgggaaggaatacaaatgtaaggtctcaaacaaagggctcccggcacccattgagaagacaatttccaaaaccaagggacagcccagggaaccccaagtgtatacgctgcccccaagccgggaggaaatgacgaaaaatcaggtcagcctcacgtgtctcgtaaagggattttacccgtcggacatcgcggtggagtgggagtcaaatggacagcccgaaaacaactataagaccacaccaccgatgctcgactccgacggaagcttctttttgtactcgaaactgacggtggacaaatcgcgctggcaacaggggaatgtctttagctgctcggtcatgcacgaggccctccacaatcattacactcagaaaagcttgtcgctctcgccgggtaaaggtggtggtggtggtctgccgggttgtaaatgggacctgctgatcaaacagtgggtttgtgacccgctgggatccggttctgctactggtggttccggctccgtcgcaagctctggttcaggcagtgcgactcatctgctgccgggttgtaaatgggacctgctgatcaaacagtgggtttgtgacccgctg

SEQ ID NO: 56 - DNA, 1533 bp, Artificial Sequence
  source: /note="Description of Artificial Sequence: Synthetic polynucleotide"
gaggtgcagctggtggagtctgggggaggcttggtccagcctggggggtccctgagactctcctgtgcagcttctggatttacctttagtagttattggatgagttgggtccgccaggctccagggaaagggctggagtgggtggcctacataaagcaagatggaaatgagaaatactatgtggactctgtgaagggccgattcaccatctccagagacaacgccaagaactcattgtatctgcaaatgaacagcctgagagccgaggacacggctgtgtattactgtgcgagggaagggatactttggttcggggacttaccgacgttctggggccagggaaccctggtcaccgtctctagtgcctccaccaagggcccatcggtcttccccctggcgccctgctccaggagcacctccgagagcacagcggccctgggctgcctggtcaaggactacttccccgaaccggtgacggtgtcgtggaactcaggcgctctgaccagcggcgtgcacaccttcccagctgtcctacagtcctcaggactctactccctcagcagcgtggtaacggtgccctcctcaaatttcgggacgcagacatatacatgcaatgtggatcataagccttccaacacgaaggtggacaagactgtggagcggaagtgttgcgtcgagtgcccaccgtgtcccgctcctccggtcgctggcccatcagtatttctcttccctcccaagccaaaagatacactcatgatctcaagaaccccagaagtgacttgtgtggtcgtggacgtgtcgcatgaggatccggaggtgcagtttaactggtatgtggatggcgtagaagtccacaacgccaagaccaagcctagagaggaacaattcaactcgacgttcagggtggtcagcgtgttgacagtagtccaccaggactggcttaatgggaaggaatacaaatgtaaggtctcaaacaaagggctcccggcacccattgagaagacaatttccaaaaccaagggacagcccagggaaccccaagtgtatacgctgcccccaagccgggaggaaatgacgaaaaatcaggtcagcctcacgtgtctcgtaaagggattttacccgtcggacatcgcggtggagtgggagtcaaatggacagcccgaaaacaactataagaccacaccaccgatgctcgactccgacggaagcttctttttgtactcgaaactgacggtggacaaatcgcgctggcaacaggggaatgtctttagctgctcggtcatgcacgaggccctccacaatcattacactcagaaaagcttgtcgctctcgccgggtaaaggtggtggtggtggtctgccgggttgtaaatgggacctgctgatcaaacagtgggtttgtgacccgctgggatccggttctgctactggtggttccggctcctcggcaagctctggttcaggcagtgcgactcatctgctgccgggttgtaaatgggacctgctgatcaaacagtgggtttgtgacccgctg

SEQ ID NO: 57 - DNA, 642 bp, Artificial Sequence
  source: /note="Description of Artificial Sequence: Synthetic polynucleotide"
gacatccagatgacccagtctccatcctcactgtctgcatctgtaggagacagagtcaccatcacttgtcgggcgagtcagggtattagcaactggttagcctggtatcagcagaaaccagagaaagcccctaagtccctgatctatgctgcatccagtttgcaaagtggggtcccatcaaggttcagcggcagtggatctgggacagatttcactctcaccatcagcagcctgcagcctgaagattttgcaacttattactgccaacagtatgatagttaccctcggacgttcggccaagggaccaaggtggaaatcaaacgaactgtggctgcaccatctgtcttcatcttcccgccatctgatgagcagttgaaatctggaactgcctctgttgtgtgcctgctgaataacttctatcccagagaggccaaagtacagtggaaggtggataacgccctccaatcgggtaactcccaggagagtgtcacagagcaggacagcaaggacagcacctacagcctcagcagcaccctgacgctgagcaaagcagactacgagaaacacaaagtctacgcctgcgaagtcacccatcagggcctgagctcgcccgtcacaaagagcttcaacaggggagagtgt

SEQ ID NO: 58 - DNA, 69 bp, Artificial Sequence
  source: /note="Description of Artificial Sequence: Synthetic oligonucleotide"
ggaagcggctcggcgacgggtgggtcggggtcgggtgcgtccagcggatcgggctcggccactgggtca

SEQ ID NO: 59 - DNA, 1341 bp, Artificial Sequence
  source: /note="Description of Artificial Sequence: Synthetic polynucleotide"
gaggtgcagctggtggagtctgggggaggcttggtccagcctggggggtccctgagactctcctgtgcagcttctggatttacctttagtagttattggatgagttgggtccgccaggctccagggaaagggctggagtgggtggcctacataaagcaagatggaaatgagaaatactatgtggactctgtgaagggccgattcaccatctccagagacaacgccaagaactcattgtatctgcaaatgaacagcctgagagccgaggacacggctgtgtattactgtgcgagggaagggatactttggttcggggacttaccgacgttctggggccagggaaccctggtcaccgtctctagtgcctccaccaagggcccatcggtcttccccctggcgccctgctccaggagcacctccgagagcacagcggccctgggctgcctggtcaaggactacttccccgaaccggtgacggtgtcgtggaactcaggcgctctgaccagcggcgtgcacaccttcccagctgtcctacagtcctcaggactctactccctcagcagcgtggtaacggtgccctcctcaaatttcgggacgcagacatatacatgcaatgtggatcataagccttccaacacgaaggtggacaagactgtggagcggaagtgttgcgtcgagtgcccaccgtgtcccgctcctccggtcgctggcccatcagtatttctcttccctcccaagccaaaagatacactcatgatctcaagaaccccagaagtgacttgtgtggtcgtggacgtgtcgcatgaggatccggaggtgcagtttaactggtatgtggatggcgtagaagtccacaacgccaagaccaagcctagagaggaacaattcaactcgacgttcagggtggtcagcgtgttgacagtagtccaccaggactggcttaatgggaaggaatacaaatgtaaggtctcaaacaaagggctcccggcacccattgagaagacaatttccaaaaccaagggacagcccagggaaccccaagtgtatacgctgcccccaagccgggaggaaatgacgaaaaatcaggtcagcctcacgtgtctcgtaaagggattttacccgtcggacatcgcggtggagtgggagtcaaatggacagcccgaaaacaactataagaccacaccaccgatgctcgactccgacggaagcttctttttgtactcgaaactgacggtggacaaatcgcgctggcaacaggggaatgtctttagctgctcggtcatgcacgaggccctccacaatcattacactcagaaaagcttgtcgctctcgccgggtaaa

SEQ ID NO: 60 - DNA, 1524 bp, Artificial Sequence
  source: /note="Description of Artificial Sequence: Synthetic polynucleotide"
cttcccggatgcaagtgggatctgttgatcaagcaatgggtctgcgaccctctcgggtcagggtccgcgaccggtggatcggggtcgggagcgtcatcgggcagcggaagcgctacgggatcacttcccgggtgcaaatgggacctcctgatcaaacaatgggtatgtgatccgctcggtggcgaggtgcagctggtggagtctgggggaggcttggtccagcctggggggtccctgagactctcctgtgcagcttctggatttacctttagtagttattggatgagttgggtccgccaggctccagggaaagggctggagtgggtggcctacataaagcaagatggaaatgagaaatactatgtggactctgtgaagggccgattcaccatctccagagacaacgccaagaactcattgtatctgcaaatgaacagcctgagagccgaggacacggctgtgtattactgtgcgagggaagggatactttggttcggggacttaccgacgttctggggccagggaaccctggtcaccgtctctagtgcctccaccaagggcccatcggtcttccccctggcgccctgctccaggagcacctccgagagcacagcggccctgggctgcctggtcaaggactacttccccgaaccggtgacggtgtcgtggaactcaggcgctctgaccagcggcgtgcacaccttcccagctgtcctacagtcctcaggactctactccctcagcagcgtggtgaccgtgccctccagcaacttcggcacccagacctacacctgcaacgtagatcacaagcccagcaacaccaaggtggacaagacagttgagcgcaaatgttgtgtcgagtgcccaccgtgcccagcaccacctgtggcaggaccgtcagtcttcctcttccccccaaaacccaaggacaccctcatgatctcccggacccctgaggtcacgtgcgtggtggtggacgtgagccacgaagaccccgaggtccagttcaactggtacgtggacggcgtggaggtgcataatgccaagacaaagccacgggaggagcagttcaacagcacgttccgtgtggtcagcgtcctcaccgttgtgcaccaggactggctgaacggcaaggagtacaagtgcaaggtctccaacaaaggcctcccagcccccatcgagaaaaccatctccaaaaccaaagggcagccccgagaaccacaggtgtacaccctgcccccatcccgggaggagatgaccaagaaccaggtcagcctgacctgcctggtcaaaggcttctaccccagcgacatcgccgtggagtgggagagcaatgggcagccggagaacaactacaagaccacacctcccatgctggactccgacggctccttcttcctctacagcaagctcaccgtggacaagagcaggtggcagcaggggaacgtcttctcatgctccgtgatgcatgaggctctgcacaaccactacacgcagaagagcctctccctgtctccgggtaaa

SEQ ID NO: 61 - DNA, 825 bp, Artificial Sequence
  source: /note="Description of Artificial Sequence: Synthetic polynucleotide"
ctccctgggtgcaaatgggacctgttgattaagcagtgggtctgcgaccctctcggatcgggaagcgcaactgggggttcaggctcaggggctagctccggatcggggtcggccacagggtcgctccccggatgtaagtgggaccttttgattaaacagtgggtgtgcgatccacttggaggtgatatccagatgacacagtcaccctcgtcgttgagcgccagcgtgggagatagagtgacgatcacctgtcgagccagccagggcatctccaactggcttgcgtggtaccaacaaaagcccgagaaggcaccgaaatcgctgatctacgcggcgtcgtcactgcagtcgggtgtaccgtcgcggtttagcgggtccgggtccggaacggacttcacgctcacgatttcctcattgcagccggaagattttgcgacttattactgtcagcaatatgactcatatccccgcacattcggtcagggaaccaaggtcgagatcaaacgtacggtggctgcaccatctgtcttcatcttcccgccatctgatgagcagttgaaatctggaactgcctctgttgtgtgcctgctgaataacttctatcccagagaggccaaagtacagtggaaggtggataacgccctccaatcgggtaactcccaggagagtgtcacagagcaggacagcaaggacagcacctacagcctcagcagcaccctgacgctgagcaaagcagactacgagaaacacaaagtctacgcctgcgaagtcacccatcagggcctgagctcgcccgtcacaaagagcttcaacaggggagagtgt

SEQ ID NO: 62 - DNA, 1533 bp, Artificial Sequence
  source: /note="Description of Artificial Sequence: Synthetic polynucleotide"
gaggtgcagctggtggagtctgggggaggcttggtccagcctggggggtccctgagactctcctgtgcagcttctggatttacctttagtagttattggatgagttgggtccgccaggctccagggaaagggctggagtgggtggcctacataaagcaagatggaaatgagaaatactatgtggactctgtgaagggccgattcaccatctccagagacaacgccaagaactcattgtatctgcaaatgaacagcctgagagccgaggacacggctgtgtattactgtgcgagggaagggatactttggttcggggacttaccgacgttctggggccagggaaccctggtcaccgtctctagtgcctccaccaagggcccatcggtcttccccctggcgccctgctccaggagcacctccgagagcacagcggccctgggctgcctggtcaaggactacttccccgaaccggtgacggtgtcgtggaactcaggcgctctgaccagcggcgtgcacaccttcccagctgtcctacagtcctcaggactctactccctcagcagcgtggtaacggtgccctcctcaaatttcgggacgcagacatatacatgcaatgtggatcataagccttccaacacgaaggtggacaagactgtggagcggaagtgttgcgtcgagtgcccaccgtgtcccgctcctccggtcgctggcccatcagtatttctcttccctcccaagccaaaagatacactcatgatctcaagaaccccagaagtgacttgtgtggtcgtggacgtgtcgcatgaggatccggaggtgcagtttaactggtatgtggatggcgtagaagtccacaacgccaagaccaagcctagagaggaacaattcaactcgacgttcagggtggtcagcgtgttgacagtagtccaccaggactggcttaatgggaaggaatacaaatgtaaggtctcaaacaaagggctcccggcacccattgagaagacaatttccaaaaccaagggacagcccagggaaccccaagtgtatacgctgcccccaagccgggaggaaatgacgaaaaatcaggtcagcctcacgtgtctcgtaaagggattttacccgtcggacatcgcggtggagtgggagtcaaatggacagcccgaaaacaactacaaaacgaccccacctatgctcgattcggacggcagcttctttttgtattcaaagttgacagtggacaaatcgcgatggcagcagggcaacgtcttctcatgttcagtaatgcatgaggcccttcacaaccactacacgcagaagtccctctcattgtcgccgggtgggggtggaggactgcccgggtgcaagtgggacctcttgatcaaacagtgggtatgcgaccctttgggagggggtgggtcaggagggggaggttccggtggaggtggttccgggggaggcggatcaggaggtggaggatcgttgcccggctgtaagtgggatctgctgatcaagcagtgggtctgtgatcctttg

SEQ ID NO: 63 - DNA, 1530 bp, Artificial Sequence
  source: /note="Description of Artificial Sequence: Synthetic polynucleotide"
gaggtgcagctggtggagtctgggggaggcttggtccagcctggggggtccctgagactctcctgtgcagcttctggatttacctttagtagttattggatgagttgggtccgccaggctccagggaaagggctggagtgggtggcctacataaagcaagatggaaatgagaaatactatgtggactctgtgaagggccgattcaccatctccagagacaacgccaagaactcattgtatctgcaaatgaacagcctgagagccgaggacacggctgtgtattactgtgcgagggaagggatactttggttcggggacttaccgacgttctggggccagggaaccctggtcaccgtctctagtgcctccaccaagggcccatcggtcttccccctggcgccctgctccaggagcacctccgagagcacagcggccctgggctgcctggtcaaggactacttccccgaaccggtgacggtgtcgtggaactcaggcgctctgaccagcggcgtgcacaccttcccagctgtcctacagtcctcaggactctactccctcagcagcgtggtgaccgtgccctccagcaacttcggcacccagacctacacctgcaacgtagatcacaagcccagcaacaccaaggtggacaagacagttgagcgcaaatgttgtgtcgagtgcccaccgtgcccagcaccacctgtggcaggaccgtcagtcttcctcttccccccaaaacccaaggacaccctcatgatctcccggacccctgaggtcacgtgcgtggtggtggacgtgagccacgaagaccccgaggtccagttcaactggtacgtggacggcgtggaggtgcataatgccaagacaaagccacgggaggagcagttcaacagcacgttccgtgtggtcagcgtcctcaccgttgtgcaccaggactggctgaacggcaaggagtacaagtgcaaggtctccaacaaaggcctcccagcccccatcgagaaaaccatctccaaaaccaaagggcagccccgagaaccacaggtgtacaccctgccaccttcgcgggaggaaatgggaggactccccgggtgcaagtgggatcttcttatcaaacagtgggtatgcgacccgctggggtcagggtcagcgacaggtggatcgggtagcggcgcatcgagcggatcagggtccgcgacgggctcacttcccggatgcaaatgggacctcttgattaagcagtgggtgtgtgacccgttgggtggaacgaagaatcaggtctcgttgacgtgtctggtgaaggggttttatccctcggatatcgctgtcgagtgggagtcgaatggacagcccgaaaacaactacaagaccaccccgcctatgctggactccgatggttccttctttttgtactcgaaactgactgtggataagagcaggtggcagcaagggaatgtattctcgtgttccgtcatgcacgaagccctccataaccactatacacaaaaatcgctttcacttagcccgggaaaa

SEQ ID NO: 64 - DNA, 1470 bp, Artificial Sequence
  source: /note="Description of Artificial Sequence: Synthetic polynucleotide"
gaggtgcagctggtggagtctgggggaggcttggtccagcctggggggtccctgagactctcctgtgcagcttctggatttacctttagtagttattggatgagttgggtccgccaggctccagggaaagggctggagtgggtggcctacataaagcaagatggaaatgagaaatactatgtggactctgtgaagggccgattcaccatctccagagacaacgccaagaactcattgtatctgcaaatgaacagcctgagagccgaggacacggctgtgtattactgtgcgagggaagggatactttggttcggggacttaccgacgttctggggccagggaaccctggtcaccgtctctagtgcctccaccaagggcccatcggtcttccccctggcgccctgctccaggagcacctccgagagcacagcggccctgggctgcctggtcaaggactacttccccgaaccggtgacggtgtcgtggaactcaggcgctctgaccagcggcgtgcacaccttcccagctgtcctacagtcctcaggactctactccctcagcagcgtggtgaccgtgccctccagcaacttcggcacccagacctacacctgcaacgtagatcacaagcccagcaacaccaaggtggacaagacagttgagcgcaaatgttgtgtcgagtgcccaccgtgcccagcaccacctgtggcaggaccgtcagtcttcctcttccccccaaaacccaaggacaccctcatgatctcccggacccctgaggtcacgtgcgtggtggtggacgtgagccacgaagaccccgaggtccagttcaactggtacgtggacggcgtggaggtgcataatgccaagacaaagccacgggaggagcagttcaacagcacgttccgtgtggtcagcgtcctcaccgttgtgcaccaggactggctgaacggcaaggagtacaagtgcaaggtctccaacaaaggcctcccagcccccatcgagaaaaccatctccaaaaccaaagggcagccccgagaaccacaggtgtacaccctgccgccctcgagagaagagatgggcgggttgccggggtgtaagtgggacttgctgattaaacaatgggtgtgcgaccctctgggcggtaccaagaatcaggtctcactgacatgtctcgtaaaaggtttttacccgtcagatatcgcggtcgagtgggaatccaacggacaacccgagaataactacaagacgactcccccaatgctcgattcggatggatccttcttcctttatagcaaacttacagtagacaaatcacggtggcagcaggggaacgtgtttagctgttcggtgatgcacgaagccttgcataatcactatacgcagaagtcgctttccctgtcgccgggagggggaggtgggctccctggatgcaagtgggatcttttgatcaagcagtgggtctgcgaccccctc

SEQ ID NO: 65 - DNA, 1473 bp, Artificial Sequence
  source: /note="Description of Artificial Sequence: Synthetic polynucleotide"
gaggtgcagctggtggagtctgggggaggcttggtccagcctggggggtccctgagactctcctgtgcagcttctggatttacctttagtagttattggatgagttgggtccgccaggctccagggaaagggctggagtgggtggcctacataaagcaagatggaaatgagaaatactatgtggactctgtgaagggccgattcaccatctccagagacaacgccaagaactcattgtatctgcaaatgaacagcctgagagccgaggacacggctgtgtattactgtgcgagggaagggatactttggttcggggacttaccgacgttctggggccagggaaccctggtcaccgtctctagtgcctccaccaagggcccatcggtcttccccctggcgccctgctccaggagcacctccgagagcacagcggccctgggctgcctggtcaaggactacttccccgaaccggtgacggtgtcgtggaactcaggcgctctgaccagcggcgtgcacaccttcccagctgtcctacagtcctcaggactctactccctcagcagcgtggtgaccgtgccctccagcaacttcggcacccagacctacacctgcaacgtagatcacaagcccagcaacaccaaggtggacaagacagttgagcgcaaatgttgtgtcgagtgcccaccgtgcccagcaccacctgtggcaggaccgtcagtcttcctcttccccccaaaacccaaggacaccctcatgatctcccggacccctgaggtcacgtgcgtggtggtggatgtaagccatgggggactgcctggatgcaagtgggatcttctcattaagcaatgggtctgtgaccctttgggcggagaggacccggaagtccagttcaactggtacgtggacggcgtggaggtgcataatgccaagacaaagccacgggaggagcagttcaacagcacgttccgtgtggtcagcgtcctcaccgttgtgcaccaggactggctgaacggcaaggagtacaagtgcaaggtctccaacaaaggcctcccagcccccatcgagaaaaccatctccaaaaccaaagggcagccccgagaaccacaggtgtacaccctgccgccctcgagagaagagatgggcgggttgccggggtgtaagtgggacttgctgattaaacaatgggtgtgcgaccctctgggcggtaccaagaatcaggtctcactgacatgtctcgtaaaaggtttttacccgtcagatatcgcggtcgagtgggaatccaacggacaacccgagaataactacaagacgactcccccaatgctcgattcggatggatccttcttcctttatagcaaacttacagtagacaaatcacggtggcagcaggggaacgtgtttagctgttcggtgatgcacgaagccttgcataatcactatacgcagaagtcgctttccctgtctccgggtaaa

SEQ ID NO: 66 - DNA, 879 bp, Artificial Sequence
  source: /note="Description of Artificial Sequence: Synthetic polynucleotide"
atgcttccaggttgtaaatgggatcttcttattaaacaatgggtttgtgatccacttggttctggttctgctactggtggttccggctccaccgcaagctctggttcaggttctgctactcatatgctgccgggttgtaaatgggacctgctgatcaaacagtgggtttgtgacccgctgggtggaggcggtggggtcgacaaaactcacacatgtccaccttgtccagctccggaactcctggggggaccgtcagtcttcctcttccccccaaaacccaaggacaccctcatgatctcccggacccctgaggtcacatgcgtggtggtggacgtgagccacgaagaccctgaggtcaagttcaactggtacgtggacggcgtggaggtgcataatgccaagacaaagccgcgggaggagcagtacaacagcacgtaccgtgtggtcagcgtcctcaccgtcctgcaccaggactggctgaatggcaaggagtacaagtgcaaggtctccaacaaagccctcccagcccccatcgagaaaaccatctccaaagccaaagggcagccccgagaaccacaggtgtacaccctgcccccatcccgggatgagctgaccaagaaccaggtcagcctgacctgcctggtcaaaggcttctatcccagcgacatcgccgtggagtgggagagcaatgggcagccggagaacaactacaagaccacgcctcccgtgctggactccgacggctccttcttcctctacagcaagctcaccgtggacaagagcaggtggcagcaggggaacgtcttctcatgctccgtgatgcatgaggctctgcacaaccactacacgcagaagagcctctccctgtctccgggtaaa

SEQ ID NO: 67 - DNA, 696 bp, Homo sapiens
gagcccaaatcttgtgacaaaactcacacatgcccaccgtgcccagcacctgaactcctggggggaccgtcagtcttcctcttccccccaaaacccaaggacaccctcatgatctcccggacccctgaggtcacatgcgtggtggtggacgtgagccacgaagaccctgaggtcaagttcaactggtacgtggacggcgtggaggtgcataatgccaagacaaagccgcgggaggagcagtacaacagcacgtaccgtgtggtcagcgtcctcaccgtcctgcaccaggactggctgaatggcaaggagtacaagtgcaaggtctccaacaaagccctcccagcccccatcgagaaaaccatctccaaagccaaagggcagccccgagaaccacaggtgtacaccctgcccccatcccgggatgagctgaccaagaaccaggtcagcctgacctgcctggtcaaaggcttctatcccagcgacatcgccgtggagtgggagagcaatgggcagccggagaacaactacaagaccacgcctcccgtgctggactccgacggctccttcttcctctatagcaagctcaccgtggacaagagcaggtggcagcaggggaacgtcttctcatgctccgtgatgcatgaggctctgcacaaccactacacgcagaagagcctctccctgtctccgggtaaa

SEQ ID NO: 68 - DNA, 684 bp, Homo sapiens
gagcgcaaatgttgtgtcgagtgcccaccgtgcccagcaccacctgtggcaggaccgtcagtcttcctcttccccccaaaacccaaggacaccctcatgatctcccggacccctgaggtcacgtgcgtggtggtggacgtgagccacgaagaccccgaggtccagttcaactggtacgtggacggcgtggaggtgcataatgccaagacaaagccacgggaggagcagttcaacagcacgttccgtgtggtcagcgtcctcaccgttgtgcaccaggactggctgaacggcaaggagtacaagtgcaaggtctccaacaaaggcctcccagcccccatcgagaaaaccatctccaaaaccaaagggcagccccgagaaccacaggtgtacaccctgcccccatcccgggaggagatgaccaagaaccaggtcagcctgacctgcctggtcaaaggcttctaccccagcgacatcgccgtggagtgggagagcaatgggcagccggagaacaactacaagaccacacctcccatgctggactccgacggctccttcttcctctacagcaagctcaccgtggacaagagcaggtggcagcaggggaacgtcttctcatgctccgtgatgcatgaggctctgcacaaccactacacgcagaagagcctctccctgtctccgggtaaa

SEQ ID NO: 69 - DNA, 837 bp, Homo sapiens
gagctcaaaaccccacttggtgacacaactcacacatgcccacggtgcccagagcccaaatcttgtgacacacctcccccgtgcccacggtgcccagagcccaaatcttgtgacacacctcccccgtgcccacggtgcccagagcccaaatcttgtgacacacctcccccatgcccacggtgcccagcacctgaactcctgggaggaccgtcagtcttcctcttccccccaaaacccaaggatacccttatgatttcccggacccctgaggtcacgtgcgtggtggtggacgtgagccacgaagaccccgaggtccagttcaagtggtacgtggacggcgtggaggtgcataatgccaagacaaagccgcgggaggagcagttcaacagcacgttccgtgtggtcagcgtcctcaccgtcctgcaccaggactggctgaacggcaaggagtacaagtgcaaggtctccaacaaagccctcccagcccccatcgagaaaaccatctccaaaaccaaaggacagccccgagaaccacaggtgtacaccctgcccccatcccgggaggagatgaccaagaaccaggtcagcctgacctgcctggtcaaaggcttctaccccagcgacatcgccgtggagtgggagagcagcgggcagccggagaacaactacaacaccacgcctcccatgctggactccgacggctccttcttcctctacagcaagctcaccgtggacaagagcaggtggcagcaggggaacatcttctcatgctccgtgatgcatgaggctctgcacaaccgcttcacgcagaagagcctctccctgtctccgggtaaa

SEQ ID NO: 70 - DNA, 687 bp, Homo sapiens
gagtccaaatatggtcccccatgcccatcatgcccagcacctgagttcctggggggaccatcagtcttcctgttccccccaaaacccaaggacactctcatgatctcccggacccctgaggtcacgtgcgtggtggtggacgtgagccaggaagaccccgaggtccagttcaactggtacgtggatggcgtggaggtgcataatgccaagacaaagccgcgggaggagcagttcaacagcacgtaccgtgtggtcagcgtcctcaccgtcctgcaccaggactggctgaacggcaaggagtacaagtgcaaggtctccaacaaaggcctcccgtcctccatcgagaaaaccatctccaaagccaaagggcagccccgagagccacaggtgtacaccctgcccccatcccaggaggagatgaccaagaaccaggtcagcctgacctgcctggtcaaaggcttctaccccagcgacatcgccgtggagtgggagagcaatgggcagccggagaacaactacaagaccacgcctcccgtgctggactccgacggctccttcttcctctacagcaggctaaccgtggacaagagcaggtggcaggaggggaatgtcttctcatgctccgtgatgcatgaggctctgcacaaccactacacacagaagagcctctccctgtctctgggtaaa

SEQ ID NO: 71 - protein, 25 aa, Artificial Sequence
  source: /note="Description of Artificial Sequence: Synthetic peptide"
GGGGSGGGGSGGGGSGGGGSGGGGS

SEQ ID NO: 72 - protein, 5 aa, Artificial Sequence
  source: /note="Description of Artificial Sequence: Synthetic peptide"
GGGGS